European Patent Application EP 4 209 590 A1, published July 12, 2023. Title: DUCHENNE MUSCULAR DYSTROPHY-RELATED EXONIC SPLICING ENHANCER, sgRNA AND GENE EDITING TOOL, AND APPLICATIONS. Applicant: WESTLAKE UNIVERSITY. The sequence listing filed with the application follows.

SEQUENCE LISTING (24 sequences)

SEQ ID NO: 1 - protein, 1420 aa, Artificial Sequence
  Amino acid sequence of fusion protein of AID-Cas9 mutant
MDYKDHDGDYKDHDIDYKDDDDKMAPKKKRKVGIHGVPAAMDSLLMNRREFLYQFKNVRWAKGRRETYLCYVVKRRDSATSFSLDFGYLRNKNGCHVELLFLRYISDWDLDPGRCYRVTWFISWSPCYDCARHVADFLRGNPNLSLRIFTARLYFCEDRKAEPEGLRRLHRAGVQIAIMTFKDYFYCWNTFVENHGRTFKAWEGLHENSVRLSRQLRRILLPSGSETPGTSESATPESGKRNYILGLAIGITSVGYGIIDYETRDVIDAGVRLFKEANVENNEGRRSKRGARRLKRRRRHRIQRVKKLLFDYNLLTDHSELSGINPYEARVKGLSQKLSEEEFSAALLHLAKRRGVHNVNEVEEDTGNELSTKEQISRNSKALEEKYVAELQLERLKKDGEVRGSINRFKTSDYVKEAKQLLKVQKAYHQLDQSFIDTYIDLLETRRTYYEGPGEGSPFGWKDIKEWYEMLMGHCTYFPEELRSVKYAYNADLYNALNDLNNLVITRDENEKLEYYEKFQIIENVFKQKKKPTLKQIAKEILVNEEDIKGYRVTSTGKPEFTNLKVYHDIKDITARKEIIENAELLDQIAKILTIYQSSEDIQEELTNLNSELTQEEIEQISNLKGYTGTHNLSLKAINLILDELWHTNDNQIAIFNRLKLVPKKVDLSQQKEIPTTLVDDFILSPVVKRSFIQSIKVINAIIKKYGLPNDIIIELAREKNSKDAQKMINEMQKRNRQTNERIEEIIRTTGKENAKYLIEKIKLHDMQEGKCLYSLEAIPLEDLLNNPFNYEVDHIIPRSVSFDNSFNNKVLVKQEENSKKGNRTPFQYLSSSDSKISYETFKKHILNLAKGKGRISKTKKEYLLEERDINRFSVQKDFINRNLVDTRYATRGLMNLLRSYFRVNNLDVKVKSINGGFTSFLRRKWKFKKERNKGYKHHAEDALIIANADFIFKEWKKLDKAKKVMENQMFEEKQAESMPEIETEQEYKEIFITPHQIKHIKDFKDYKYSHRVDKKPNRKLINDTLYSTRKDDKGNTLIVNNLNGLYDKDNDKLKKLINKSPEKLLMYHHDPQTYQKLKLIMEQYGDEKNPLYKYYEETGNYLTKYSKKDNGPVIKKIKYYGNKLNAHLDITDDYPNSRNKVVKLSLKPYRFDVYLDNGVYKFVTVKNLDVIKKENYYEVNSKCYEEAKKLKKISNQAEFIASFYKNDLIKINGELYRVIGVNNDLLNRIEVNMIDITYREYLENMNDKRPPHIIKTIASKTQSIKKYSTDILGNLYEVKSKKHPQIIKKGGSSGGSTNLSDIIEKETGKQLVIQESILMLPEEVEEVIGNKPESDILVHTAYDESTDENVMLLTSDAPEYKPWALVIQDSNGENKIKMLSGGSPKKKRKVGSYPYDVPDYAYPYDVPDYAYPYDVPDYA

SEQ ID NO: 2 - DNA, 4263 bp, Artificial Sequence
  Nucleotide sequence of fusion protein of AID-Cas9 mutant
atggactataaggaccacgacggagactacaaggatcatgatattgattacaaagacgatgacgataagatggccccaaagaagaagcggaaggtcggtatccacggagtcccagcagccatggacagcctcttgatgaaccggagggagtttctttaccaattcaaaaatgtccgctgggctaagggtcggcgtgagacctacctgtgctacgtagtgaagaggcgtgacagtgctacatccttttcactggactttggttatcttcgcaataagaacggctgccacgtggaattgctcttcctccgctacatctcggactgggacctagaccctggccgctgctaccgcgtcacctggttcatctcctggagcccctgctacgactgtgcccgacatgtggccgactttctgcgagggaaccccaacctcagtctgaggatcttcaccgcgcgcctctacttctgtgaggaccgcaaggctgagcccgaggggctgcggcggctgcaccgcgccggggtgcaaatagccatcatgaccttcaaagattatttttactgctggaatacttttgtagaaaaccatggaagaactttcaaagcctgggaagggctgcatgaaaattcagttcgtctatccagacagcttcggcgcatccttttgcccagcggcagcgagactcccgggacctcagagtccgccacacccgaaagcggcaagaggaactacatcctgggcctggccatcggcatcaccagcgtgggctacggcatcatcgactacgagaccagggacgtgatcgacgccggcgtgaggctgttcaaggaggccaacgtggagaacaacgagggcaggaggagcaagaggggcgccaggaggctgaagaggaggaggaggcacaggatccagagggtgaagaagctgctgttcgactacaacctgctgaccgaccacagcgagctgagcggcatcaacccttacgaggccagggtgaagggcctgagccagaagctgagcgaggaggagttcagcgccgccctgctgcacctggccaagaggaggggcgtgcacaacgtgaacgaggtggaggaggacaccggcaacgagctgagcaccaaggagcagatcagcaggaacagcaaggccctggaggagaagtacgtggccgagctgcagctggagaggctgaagaaggacggcgaggtgaggggcagcatcaacaggttcaagaccagcgactacgtgaaggaggccaagcagctgctgaaggtgcagaaggcctaccaccagctggaccagagcttcatcgacacctacatcgacctgctggagaccaggaggacctactacgagggccctggcgagggcagccctttcggctggaaggacatcaaggagtggtacgagatgctgatgggccactgcacctacttccctgaggagctgaggagcgtgaagtacgcctacaacgccgacctgtacaacgccctgaacgacctgaacaacctggtgatcaccagggacgagaacgagaagctggagtactacgagaagttccagatcatcgagaacgtgttcaagcagaagaagaagcctaccctgaagcagatcgccaaggagatcctggtgaacgaggaggacatcaagggctacagggtgaccagcaccggcaagcctgagttcaccaacctgaaggtgtaccacgacatcaaggacatcaccgccaggaaggagatcatcgagaacgccgagctgctggaccagatcgccaagatcctgaccatctaccagagcagcgaggacatccaggaggagctgaccaacctgaacagcgagctgacccaggaggagatcgagcagatcagcaacctgaagggctacaccggcacccacaacctgagcctgaaggccatcaacctgatcctggacgagctgtggcacaccaacgacaaccagatcgccatcttcaacaggctgaagctggtgcctaagaaggtggacctgagccagcagaaggagatccctaccaccctggtggacgacttcatcctgagccctgtggtgaagaggagcttcatccagagcatcaaggtgatcaacgccatcatcaagaagtacggcctgcctaacgacatcatcatcgagctggccagggagaagaacagcaaggacgcccagaagatgatcaacgagatgcagaagaggaacaggcagaccaacgagaggatcgaggagatcatcaggaccaccggcaaggagaacgccaagtacctgatcgagaagatcaagctgcacgacatgcaggagggcaagtgcctgtacagcctggaggccatccctctggaggacctgctgaacaaccctttcaactacgaggtggaccacatcatccctaggagcgtgagcttcgacaacagcttcaacaacaaggtgctggtgaagcaggaggagaacagcaagaagggcaacaggacccctttccagtacctgagcagcagcgacagcaagatcagctacgagaccttcaagaagcacatcctgaacctggccaagggcaagggcaggatcagcaagaccaagaaggagtacctgctggaggagagggacatcaacaggttcagcgtgcagaaggacttcatcaacaggaacctggtggacaccaggtacgccaccaggggcctgatgaacctgctgaggagctacttcagggtgaacaacctggacgtgaaggtgaagagcatcaacggcggcttcaccagcttcctgaggaggaagtggaagttcaagaaggagaggaacaagggctacaagcaccacgccgaggacgccctgatcatcgccaacgccgacttcatcttcaaggagtggaagaagctggacaaggccaagaaggtgatggagaaccagatgttcgaggagaagcaggccgagagcatgcctgagatcgagaccgagcaggagtacaaggagatcttcatcacccctcaccagatcaagcacatcaaggacttcaaggactacaagtacagccacagggtggacaagaagcctaacaggaagctgatcaacgacaccctgtacagcaccaggaaggacgacaagggcaacaccctgatcgtgaacaacctgaacggcctgtacgacaaggacaacgacaagctgaagaagctgatcaacaagagccctgagaagctgctgatgtaccaccacgaccctcagacctaccagaagctgaagctgatcatggagcagtacggcgacgagaagaaccctctgtacaagtactacgaggagaccggcaactacctgaccaagtacagcaagaaggacaacggccctgtgatcaagaagatcaagtactacggcaacaagctgaacgcccacctggacatcaccgacgactaccctaacagcaggaacaaggtggtgaagctgagcctgaagccttacaggttcgacgtgtacctggacaacggcgtgtacaagttcgtgaccgtgaagaacctggacgtgatcaagaaggagaactactacgaggtgaacagcaagtgctacgaggaggccaagaagctgaagaagatcagcaaccaggccgagttcatcgccagcttctacaagaacgacctgatcaagatcaacggcgagctgtacagggtgatcggcgtgaacaacgacctgctgaacaggatcgaggtgaacatgatcgacatcacctacagggagtacctggagaacatgaacgacaagaggcctcctcacatcatcaagaccatcgccagcaagacccagagcatcaagaagtacagcaccgacatcctgggcaacctgtacgaggtgaagagcaagaagcaccctcagatcatcaagaagggcggcagcagcggcggcagcaccaacctgagcgacatcatcgagaaggagaccggtaagcaactggttatccaggaatccatcctcatgctcccagaggaggtggaagaagtcattgggaacaagccggaaagcgatatactcgtgcacaccgcctacgacgagagcaccgacgagaatgtcatgcttctgactagcgacgcccctgaatacaagccttgggctctggtcatacaggatagcaacggtgagaacaagattaagatgctctctggtggttctcccaagaagaagaggaaagtcggatcctacccatacgatgttccagattacgcttacccatacgatgttccagattacgcttacccatacgatgttccagattacgcttaa

SEQ ID NO: 3 - DNA, 7661 bp, Artificial Sequence
  Sequence of AAV plasmid vector expressing fusion protein of AID-Cas9 mutant
cctgcaggcagctgcgcgctcgctcgctcactgaggccgcccgggcgtcgggcgacctttggtcgcccggcctcagtgagcgagcgagcgcgcagagagggagtggccaactccatcactaggggttcctgcggcctctagactcgagcggccgtccgccctcggcaccattcctcacgacaccgaaatatggcgacgggtgaggaatggtggggagttatttttagagcggtgaggaatggtgggcaggcagcaggtgttgggggagttatttttagagcggggagttatttttagagcggtgaggaatggtggacaccgaaatatggcgacgggtgaggaatggtgccgtcgccatatttgggtgtcccgtccgccctcggccggggccgcattcctgggggccgggcggtgctcccgcccgcctcgataaaaggctccggggccggcggcggcccacgagctacccggaggagcgggaggcgtctctgccagcggtccgacgcgcagtcagcaccaggtaggtgggcaccgcgccgtgccgtgccgctagctaatacgactcactatagggagagccgccaccatggactataaggaccacgacggagactacaaggatcatgatattgattacaaagacgatgacgataagatggccccaaagaagaagcggaaggtcggtatccacggagtcccagcagccatggacagcctcttgatgaaccggagggagtttctttaccaattcaaaaatgtccgctgggctaagggtcggcgtgagacctacctgtgctacgtagtgaagaggcgtgacagtgctacatccttttcactggactttggttatcttcgcaataagaacggctgccacgtggaattgctcttcctccgctacatctcggactgggacctagaccctggccgctgctaccgcgtcacctggttcatctcctggagcccctgctacgactgtgcccgacatgtggccgactttctgcgagggaaccccaacctcagtctgaggatcttcaccgcgcgcctctacttctgtgaggaccgcaaggctgagcccgaggggctgcggcggctgcaccgcgccggggtgcaaatagccatcatgaccttcaaagattatttttactgctggaatacttttgtagaaaaccatggaagaactttcaaagcctgggaagggctgcatgaaaattcagttcgtctatccagacagcttcggcgcatccttttgcccagcggcagcgagactcccgggacctcagagtccgccacacccgaaagcggcaagaggaactacatcctgggcctggccatcggcatcaccagcgtgggctacggcatcatcgactacgagaccagggacgtgatcgacgccggcgtgaggctgttcaaggaggccaacgtggagaacaacgagggcaggaggagcaagaggggcgccaggaggctgaagaggaggaggaggcacaggatccagagggtgaagaagctgctgttcgactacaacctgctgaccgaccacagcgagctgagcggcatcaacccttacgaggccagggtgaagggcctgagccagaagctgagcgaggaggagttcagcgccgccctgctgcacctggccaagaggaggggcgtgcacaacgtgaacgaggtggaggaggacaccggcaacgagctgagcaccaaggagcagatcagcaggaacagcaaggccctggaggagaagtacgtggccgagctgcagctggagaggctgaagaaggacggcgaggtgaggggcagcatcaacaggttcaagaccagcgactacgtgaaggaggccaagcagctgctgaaggtgcagaaggcctaccaccagctggaccagagcttcatcgacacctacatcgacctgctggagaccaggaggacctactacgagggccctggcgagggcagccctttcggctggaaggacatcaaggagtggtacgagatgctgatgggccactgcacctacttccctgaggagctgaggagcgtgaagtacgcctacaacgccgacctgtacaacgccctgaacgacctgaacaacctggtgatcaccagggacgagaacgagaagctggagtactacgagaagttccagatcatcgagaacgtgttcaagcagaagaagaagcctaccctgaagcagatcgccaaggagatcctggtgaacgaggaggacatcaagggctacagggtgaccagcaccggcaagcctgagttcaccaacctgaaggtgtaccacgacatcaaggacatcaccgccaggaaggagatcatcgagaacgccgagctgctggaccagatcgccaagatcctgaccatctaccagagcagcgaggacatccaggaggagctgaccaacctgaacagcgagctgacccaggaggagatcgagcagatcagcaacctgaagggctacaccggcacccacaacctgagcctgaaggccatcaacctgatcctggacgagctgtggcacaccaacgacaaccagatcgccatcttcaacaggctgaagctggtgcctaagaaggtggacctgagccagcagaaggagatccctaccaccctggtggacgacttcatcctgagccctgtggtgaagaggagcttcatccagagcatcaaggtgatcaacgccatcatcaagaagtacggcctgcctaacgacatcatcatcgagctggccagggagaagaacagcaaggacgcccagaagatgatcaacgagatgcagaagaggaacaggcagaccaacgagaggatcgaggagatcatcaggaccaccggcaaggagaacgccaagtacctgatcgagaagatcaagctgcacgacatgcaggagggcaagtgcctgtacagcctggaggccatccctctggaggacctgctgaacaaccctttcaactacgaggtggaccacatcatccctaggagcgtgagcttcgacaacagcttcaacaacaaggtgctggtgaagcaggaggagaacagcaagaagggcaacaggacccctttccagtacctgagcagcagcgacagcaagatcagctacgagaccttcaagaagcacatcctgaacctggccaagggcaagggcaggatcagcaagaccaagaaggagtacctgctggaggagagggacatcaacaggttcagcgtgcagaaggacttcatcaacaggaacctggtggacaccaggtacgccaccaggggcctgatgaacctgctgaggagctacttcagggtgaacaacctggacgtgaaggtgaagagcatcaacggcggcttcaccagcttcctgaggaggaagtggaagttcaagaaggagaggaacaagggctacaagcaccacgccgaggacgccctgatcatcgccaacgccgacttcatcttcaaggagtggaagaagctggacaaggccaagaaggtgatggagaaccagatgttcgaggagaagcaggccgagagcatgcctgagatcgagaccgagcaggagtacaaggagatcttcatcacccctcaccagatcaagcacatcaaggacttcaaggactacaagtacagccacagggtggacaagaagcctaacaggaagctgatcaacgacaccctgtacagcaccaggaaggacgacaagggcaacaccctgatcgtgaacaacctgaacggcctgtacgacaaggacaacgacaagctgaagaagctgatcaacaagagccctgagaagctgctgatgtaccaccacgaccctcagacctaccagaagctgaagctgatcatggagcagtacggcgacgagaagaaccctctgtacaagtactacgaggagaccggcaactacctgaccaagtacagcaagaaggacaacggccctgtgatcaagaagatcaagtactacggcaacaagctgaacgcccacctggacatcaccgacgactaccctaacagcaggaacaaggtggtgaagctgagcctgaagccttacaggttcgacgtgtacctggacaacggcgtgtacaagttcgtgaccgtgaagaacctggacgtgatcaagaaggagaactactacgaggtgaacagcaagtgctacgaggaggccaagaagctgaagaagatcagcaaccaggccgagttcatcgccagcttctacaagaacgacctgatcaagatcaacggcgagctgtacagggtgatcggcgtgaacaacgacctgctgaacaggatcgaggtgaacatgatcgacatcacctacagggagtacctggagaacatgaacgacaagaggcctcctcacatcatcaagaccatcgccagcaagacccagagcatcaagaagtacagcaccgacatcctgggcaacctgtacgaggtgaagagcaagaagcaccctcagatcatcaagaagggcggcagcagcggcggcagcaccaacctgagcgacatcatcgagaaggagaccggtaagcaactggttatccaggaatccatcctcatgctcccagaggaggtggaagaagtcattgggaacaagccggaaagcgatatactcgtgcacaccgcctacgacgagagcaccgacgagaatgtcatgcttctgactagcgacgcccctgaatacaagccttgggctctggtcatacaggatagcaacggtgagaacaagattaagatgctctctggtggttctcccaagaagaagaggaaagtcggatcctacccatacgatgttccagattacgcttacccatacgatgttccagattacgcttacccatacgatgttccagattacgcttaagaattctagcaataaaggatcgtttattttcattggaagcgtgtgttggttttttgatcaggcgcggcggccgcaggaacccctagtgatggagttggccactccctctctgcgcgctcgctcgctcactgaggccgggcgaccaaaggtcgcccgacgcccgggctttgcccgggcggcctcagtgagcgagcgagcgcgcagctgcctgcaggggcgcctgatgcggtattttctccttacgcatctgtgcggtatttcacaccgcatacgtcaaagcaaccatagtacgcgccctgtagcggcgcattaagcgcggcgggtgtggtggttacgcgcagcgtgaccgctacacttgccagcgccttagcgcccgctcctttcgctttcttcccttcctttctcgccacgttcgccggctttccccgtcaagctctaaatcgggggctccctttagggttccgatttagtgctttacggcacctcgaccccaaaaaacttgatttgggtgatggttcacgtagtgggccatcgccctgatagacggtttttcgccctttgacgttggagtccacgttctttaatagtggactcttgttccaaactggaacaacactcaactctatctcgggctattcttttgatttataagggattttgccgatttcggtctattggttaaaaaatgagctgatttaacaaaaatttaacgcgaattttaacaaaatattaacgtttacaattttatggtgcactctcagtacaatctgctctgatgccgcatagttaagccagccccgacacccgccaacacccgctgacgcgccctgacgggcttgtctgctcccggcatccgcttacagacaagctgtgaccgtctccgggagctgcatgtgtcagaggttttcaccgtcatcaccgaaacgcgcgagacgaaagggcctcgtgatacgcctatttttataggttaatgtcatgataataatggtttcttagacgtcaggtggcacttttcggggaaatgtgcgcggaacccctatttgtttatttttctaaatacattcaaatatgtatccgctcatgagacaataaccctgataaatgcttcaataatattgaaaaaggaagagtatgagtattcaacatttccgtgtcgcccttattcccttttttgcggcattttgccttcctgtttttgctcacccagaaacgctggtgaaagtaaaagatgctgaagatcagttgggtgcacgagtgggttacatcgaactggatctcaacagcggtaagatccttgagagttttcgccccgaagaacgttttccaatgatgagcacttttaaagttctgctatgtggcgcggtattatcccgtattgacgccgggcaagagcaactcggtcgccgcatacactattctcagaatgacttggttgagtactcaccagtcacagaaaagcatcttacggatggcatgacagtaagagaattatgcagtgctgccataaccatgagtgataacactgcggccaacttacttctgacaacgatcggaggaccgaaggagctaaccgcttttttgcacaacatgggggatcatgtaactcgccttgatcgttgggaaccggagctgaatgaagccataccaaacgacgagcgtgacaccacgatgcctgtagcaatggcaacaacgttgcgcaaactattaactggcgaactacttactctagcttcccggcaacaattaatagactggatggaggcggataaagttgcaggaccacttctgcgctcggcccttccggctggctggtttattgctgataaatctggagccggtgagcgtggaagccgcggtatcattgcagcactggggccagatggtaagccctcccgtatcgtagttatctacacgacggggagtcaggcaactatggatgaacgaaatagacagatcgctgagataggtgcctcactgattaagcattggtaactgtcagaccaagtttactcatatatactttagattgatttaaaacttcatttttaatttaaaaggatctaggtgaagatcctttttgataatctcatgaccaaaatcccttaacgtgagttttcgttccactgagcgtcagaccccgtagaaaagatcaaaggatcttcttgagatcctttttttctgcgcgtaatctgctgcttgcaaacaaaaaaaccaccgctaccagcggtggtttgtttgccggatcaagagctaccaactctttttccgaaggtaactggcttcagcagagcgcagataccaaatactgttcttctagtgtagccgtagttaggccaccacttcaagaactctgtagcaccgcctacatacctcgctctgctaatcctgttaccagtggctgctgccagtggcgataagtcgtgtcttaccgggttggactcaagacgatagttaccggataaggcgcagcggtcgggctgaacggggggttcgtgcacacagcccagcttggagcgaacgacctacaccgaactgagatacctacagcgtgagctatgagaaagcgccacgcttcccgaagggagaaaggcggacaggtatccggtaagcggcagggtcggaacaggagagcgcacgagggagcttccagggggaaacgcctggtatctttatagtcctgtcgggtttcgccacctctgacttgagcgtcgatttttgtgatgctcgtcaggggggcggagcctatggaaaaacgccagcaacgcggcctttttacggttcctggccttttgctggccttttgctcacatgt

SEQ ID NO: 4 - DNA, 20 bp, Artificial Sequence
  sgRNA targeting Dmd-E4 mouse mutation site
cattatttttctgtaagacc

SEQ ID NO: 5 - DNA, 5895 bp, Artificial Sequence
  Sequence of AAV vector plasmid expressing sgRNA targeting Dmd-E4 mouse mutation site
cctgcaggcagctgcgcgctcgctcgctcactgaggccgcccgggcgtcgggcgacctttggtcgcccggcctcagtgagcgagcgagcgcgcagagagggagtggccaactccatcactaggggttcctgcggcctctagactcgaggagggcctatttcccatgattccttcatatttgcatatacgatacaaggctgttagagagataattagaattaatttgactgtaaacacaaagatattagtacaaaatacgtgacgtagaaagtaataatttcttgggtagtttgcagttttaaaattatgttttaaaatggactatcatatgcttaccgtaacttgaaagtatttcgatttcttggctttatatatcttgtggaaaggacgaaacaccgcattatttttctgtaagaccgttatagtactctggaaacagaatctactataacaaggcaaaatgccgtgtttatctcgtcaacttgttggcgagattttttttttttttctagacccagctttcttgtacaaagttggcattagctagcgctaaccggtggcgcgttaagtcgacgaacgctgacgtcatcaacccgctccaaggaatcgcgggcccagtgtcactaggcgggaacacccagcgcgcgtgcgccctggcaggaagatggctgtgagggacaggggagtggcgccctgcaatatttgcatgtcgctatgtgttctgggaaatcaccataaacgtgaaatgtctttggatttgggaatcttataagttctgtatgagaccacagatctgacattatttttctgtaagaccgttatagtactctggaaacagaatctactataacaaggcaaaatgccgtgtttatctcgtcaacttgttggcgagattttttttttttctagacccagctttcttgtacaaagttggcattaaagcttatcgataccctgcagtatttagcatgccccacccatctgcaaggcattctggatagtgtcaaaacagccggaaatcaagtccgtttatctcaaactttagcattttgggaataaatgatatttgctatgctggttaaattagattttagttaaatttcctgctgaagctctagtacgataagtaacttgacctaagtgtaaagttgagatttccttcaggtttatatagcttgtgcgccgcctgggtaccagatctgacattatttttctgtaagaccgttatagtactctggaaacagaatctactataacaaggcaaaatgccgtgtttatctcgtcaacttgttggcgagatttttttttttttctagacccagctttcggtactcgcggccgccggccgtccgccctcggcaccattcctcacgacaccgaaatatggcgacgggtgaggaatggtggggagttatttttagagcggtgaggaatggtgggcaggcagcaggtgttgggggagttatttttagagcggggagttatttttagagcggtgaggaatggtggacaccgaaatatggcgacgggtgaggaatggtgccgtcgccatatttgggtgtcccgtccgccctcggccggggccgcattcctgggggccgggcggtgctcccgcccgcctcgataaaaggctccggggccggcggcggcccacgagctacccggaggagcgggaggcgtctctgccagcggtccgacgcgcagtcagcaccaggtaggtgggcaccgcgccgtgccgtgccctctggctaactaccatggtgagcaagggcgaggagctgttcaccggggtggtgcccatcctggtcgagctggacggcgacgtaaacggccacaagttcagcgtgtctggcgagggcgagggcgatgccacctacggcaagctgaccctgaagttcatctgcaccaccggcaagctgcccgtgccctggcccaccctcgtgaccaccctgacctacggcgtgcagtgcttcagccgctaccccgaccacatgaagcagcacgacttcttcaagtccgccatgcccgaaggctacgtccaggagcgcaccatcttcttcaaggacgacggcaactacaagacccgcgccgaggtgaagttcgagggcgacaccctggtgaaccgcatcgagctgaagggcatcgacttcaaggaggacggcaacatcctggggcacaagctggagtacaactacaacagccacaacgtctatatcatggccgacaagcagaagaacggcatcaaggcgaacttcaagatccgccacaacatcgaggacggcagcgtgcagctcgccgaccactaccagcagaacacccccatcggcgacggccccgtgctgctgcccgacaaccactacctgagcacccagtccgccctgagcaaagaccccaacgagaagcgcgatcacatggtcctgctggagttcgtgaccgccgccgggatcactctcggcatggacgagctgtacaagtgcgcaacaaacttctctctgctgaaacaagccggagatgtcgaagagaatcctggacccactaatctgtcagatattattgaaaaggagaccggtaagcaactggttatccaggaatccatcctcatgctcccagaggaggtggaagaagtcattgggaacaagccggaaagcgatatactcgtgcacaccgcctacgacgagagcaccgacgagaatgtcatgcttctgactagcgacgcccctgaatacaagccttgggctctggtcatacaggatagcaacggtgagaacaagattaagatgctctctggtggttctcccaagaagaagaggaaagtcggatcctacccatacgatgttccagattacgcttacccatacgatgttccagattacgcttacccatacgatgttccagattacgcttaagaattcctagagctcgctgatcagcctcgactgtgccttctagttgccagccatctgttgtttgcccctcccccgtgccttccttgaccctggaaggtgccactcccactgtcctttcctaataaaatgaggaaattgcatcgcattgtctgagtaggtgtcattctattctggggggtggggtggggcaggacagcaagggggaggattgggaagagaatagcaggcatgctggggaggaattcggccgcaggaacccctagtgatggagttggccactccctctctgcgcgctcgctcgctcactgaggccgggcgaccaaaggtcgcccgacgcccgggctttgcccgggcggcctcagtgagcgagcgagcgcgcagctgcctgcaggggcgcctgatgcggtattttctccttacgcatctgtgcggtatttcacaccgcatacgtcaaagcaaccatagtacgcgccctgtagcggcgcattaagcgcggcgggtgtggtggttacgcgcagcgtgaccgctacacttgccagcgccttagcgcccgctcctttcgctttcttcccttcctttctcgccacgttcgccggctttccccgtcaagctctaaatcgggggctccctttagggttccgatttagtgctttacggcacctcgaccccaaaaaacttgatttgggtgatggttcacgtagtgggccatcgccctgatagacggtttttcgccctttgacgttggagtccacgttctttaatagtggactcttgttccaaactggaacaacactcaactctatctcgggctattcttttgatttataagggattttgccgatttcggtctattggttaaaaaatgagctgatttaacaaaaatttaacgcgaattttaacaaaatattaacgtttacaattttatggtgcactctcagtacaatctgctctgatgccgcatagttaagccagccccgacacccgccaacacccgctgacgcgccctgacgggcttgtctgctcccggcatccgcttacagacaagctgtgaccgtctccgggagctgcatgtgtcagaggttttcaccgtcatcaccgaaacgcgcgagacgaaagggcctcgtgatacgcctatttttataggttaatgtcatgataataatggtttcttagacgtcaggtggcacttttcggggaaatgtgcgcggaacccctatttgtttatttttctaaatacattcaaatatgtatccgctcatgagacaataaccctgataaatgcttcaataatattgaaaaaggaagagtatgagtattcaacatttccgtgtcgcccttattcccttttttgcggcattttgccttcctgtttttgctcacccagaaacgctggtgaaagtaaaagatgctgaagatcagttgggtgcacgagtgggttacatcgaactggatctcaacagcggtaagatccttgagagttttcgccccgaagaacgttttccaatgatgagcacttttaaagttctgctatgtggcgcggtattatcccgtattgacgccgggcaagagcaactcggtcgccgcatacactattctcagaatgacttggttgagtactcaccagtcacagaaaagcatcttacggatggcatgacagtaagagaattatgcagtgctgccataaccatgagtgataacactgcggccaacttacttctgacaacgatcggaggaccgaaggagctaaccgcttttttgcacaacatgggggatcatgtaactcgccttgatcgttgggaaccggagctgaatgaagccataccaaacgacgagcgtgacaccacgatgcctgtagcaatggcaacaacgttgcgcaaactattaactggcgaactacttactctagcttcccggcaacaattaatagactggatggaggcggataaagttgcaggaccacttctgcgctcggcccttccggctggctggtttattgctgataaatctggagccggtgagcgtggaagccgcggtatcattgcagcactggggccagatggtaagccctcccgtatcgtagttatctacacgacggggagtcaggcaactatggatgaacgaaatagacagatcgctgagataggtgcctcactgattaagcattggtaactgtcagaccaagtttactcatatatactttagattgatttaaaacttcatttttaatttaaaaggatctaggtgaagatcctttttgataatctcatgaccaaaatcccttaacgtgagttttcgttccactgagcgtcagaccccgtagaaaagatcaaaggatcttcttgagatcctttttttctgcgcgtaatctgctgcttgcaaacaaaaaaaccaccgctaccagcggtggtttgtttgccggatcaagagctaccaactctttttccgaaggtaactggcttcagcagagcgcagataccaaatactgttcttctagtgtagccgtagttaggccaccacttcaagaactctgtagcaccgcctacatacctcgctctgctaatcctgttaccagtggctgctgccagtggcgataagtcgtgtcttaccgggttggactcaagacgatagttaccggataaggcgcagcggtcgggctgaacggggggttcgtgcacacagcccagcttggagcgaacgacctacaccgaactgagatacctacagcgtgagctatgagaaagcgccacgcttcccgaagggagaaaggcggacaggtatccggtaagcggcagggtcggaacaggagagcgcacgagggagcttccagggggaaacgcctggtatctttatagtcctgtcgggtttcgccacctctgacttgagcgtcgatttttgtgatgctcgtcaggggggcggagcctatggaaaaacgccagcaacgcggcctttttacggttcctggccttttgctggccttttgctcacatgt

SEQ ID NO: 6 - DNA, 5067 bp, Artificial Sequence
  The corresponding sequence comprising AID-Cas9 fusion protein and sgRNA targeting Dmd-E4 mouse in the one AAV vector plasmid
gcggcctctagactcgagcggccgtccgccctcggcaccattcctcacgacaccgaaatatggcgacgggtgaggaatggtggggagttatttttagagcggtgaggaatggtgggcaggcagcaggtgttgggggagttatttttagagcggggagttatttttagagcggtgaggaatggtggacaccgaaatatggcgacgggtgaggaatggtgccgtcgccatatttgggtgtcccgtccgccctcggccggggccgcattcctgggggccgggcggtgctcccgcccgcctcgataaaaggctccggggccggcggcggcccacgagctacccggaggagcgggaggcgtctctgccagcggtccgacgcgcagtcagcaccaggtaggtgggcaccgcgccgtgccgtgccgctagctaatacgactcactatagggagagccgccaccatggactataaggaccacgacggagactacaaggatcatgatattgattacaaagacgatgacgataagatggccccaaagaagaagcggaaggtcggtatccacggagtcccagcagccatggacagcctcttgatgaaccggagggagtttctttaccaattcaaaaatgtccgctgggctaagggtcggcgtgagacctacctgtgctacgtagtgaagaggcgtgacagtgctacatccttttcactggactttggttatcttcgcaataagaacggctgccacgtggaattgctcttcctccgctacatctcggactgggacctagaccctggccgctgctaccgcgtcacctggttcatctcctggagcccctgctacgactgtgcccgacatgtggccgactttctgcgagggaaccccaacctcagtctgaggatcttcaccgcgcgcctctacttctgtgaggaccgcaaggctgagcccgaggggctgcggcggctgcaccgcgccggggtgcaaatagccatcatgaccttcaaagattatttttactgctggaatacttttgtagaaaaccatggaagaactttcaaagcctgggaagggctgcatgaaaattcagttcgtctatccagacagcttcggcgcatccttttgcccagcggcagcgagactcccgggacctcagagtccgccacacccgaaagcggcaagaggaactacatcctgggcctggccatcggcatcaccagcgtgggctacggcatcatcgactacgagaccagggacgtgatcgacgccggcgtgaggctgttcaaggaggccaacgtggagaacaacgagggcaggaggagcaagaggggcgccaggaggctgaagaggaggaggaggcacaggatccagagggtgaagaagctgctgttcgactacaacctgctgaccgaccacagcgagctgagcggcatcaacccttacgaggccagggtgaagggcctgagccagaagctgagcgaggaggagttcagcgccgccctgctgcacctggccaagaggaggggcgtgcacaacgtgaacgaggtggaggaggacaccggcaacgagctgagcaccaaggagcagatcagcaggaacagcaaggccctggaggagaagtacgtggccgagctgcagctggagaggctgaagaaggacggcgaggtgaggggcagcatcaacaggttcaagaccagcgactacgtgaaggaggccaagcagctgctgaaggtgcagaaggcctaccaccagctggaccagagcttcatcgacacctacatcgacctgctggagaccaggaggacctactacgagggccctggcgagggcagccctttcggctggaaggacatcaaggagtggtacgagatgctgatgggccactgcacctacttccctgaggagctgaggagcgtgaagtacgcctacaacgccgacctgtacaacgccctgaacgacctgaacaacctggtgatcaccagggacgagaacgagaagctggagtactacgagaagttccagatcatcgagaacgtgttcaagcagaagaagaagcctaccctgaagcagatcgccaaggagatcctggtgaacgaggaggacatcaagggctacagggtgaccagcaccggcaagcctgagttcaccaacctgaaggtgtaccacgacatcaaggacatcaccgccaggaaggagatcatcgagaacgccgagctgctggaccagatcgccaagatcctgaccatctaccagagcagcgaggacatccaggaggagctgaccaacctgaacagcgagctgacccaggaggagatcgagcagatcagcaacctgaagggctacaccggcacccacaacctgagcctgaaggccatcaacctgatcctggacgagctgtggcacaccaacgacaaccagatcgccatcttcaacaggctgaagctggtgcctaagaaggtggacctgagccagcagaaggagatccctaccaccctggtggacgacttcatcctgagccctgtggtgaagaggagcttcatccagagcatcaaggtgatcaacgccatcatcaagaagtacggcctgcctaacgacatcatcatcgagctggccagggagaagaacagcaaggacgcccagaagatgatcaacgagatgcagaagaggaacaggcagaccaacgagaggatcgaggagatcatcaggaccaccggcaaggagaacgccaagtacctgatcgagaagatcaagctgcacgacatgcaggagggcaagtgcctgtacagcctggaggccatccctctggaggacctgctgaacaaccctttcaactacgaggtggaccacatcatccctaggagcgtgagcttcgacaacagcttcaacaacaaggtgctggtgaagcaggaggagaacagcaagaagggcaacaggacccctttccagtacctgagcagcagcgacagcaagatcagctacgagaccttcaagaagcacatcctgaacctggccaagggcaagggcaggatcagcaagaccaagaaggagtacctgctggaggagagggacatcaacaggttcagcgtgcagaaggacttcatcaacaggaacctggtggacaccaggtacgccaccaggggcctgatgaacctgctgaggagctacttcagggtgaacaacctggacgtgaaggtgaagagcatcaacggcggcttcaccagcttcctgaggaggaagtggaagttcaagaaggagaggaacaagggctacaagcaccacgccgaggacgccctgatcatcgccaacgccgacttcatcttcaaggagtggaagaagctggacaaggccaagaaggtgatggagaaccagatgttcgaggagaagcaggccgagagcatgcctgagatcgagaccgagcaggagtacaaggagatcttcatcacccctcaccagatcaagcacatcaaggacttcaaggactacaagtacagccacagggtggacaagaagcctaacaggaagctgatcaacgacaccctgtacagcaccaggaaggacgacaagggcaacaccctgatcgtgaacaacctgaacggcctgtacgacaaggacaacgacaagctgaagaagctgatcaacaagagccctgagaagctgctgatgtaccaccacgaccctcagacctaccagaagctgaagctgatcatggagcagtacggcgacgagaagaaccctctgtacaagtactacgaggagaccggcaactacctgaccaagtacagcaagaaggacaacggccctgtgatcaagaagatcaagtactacggcaacaagctgaacgcccacctggacatcaccgacgactaccctaacagcaggaacaaggtggtgaagctgagcctgaagccttacaggttcgacgtgtacctggacaacggcgtgtacaagttcgtgaccgtgaagaacctggacgtgatcaagaaggagaactactacgaggtgaacagcaagtgctacgaggaggccaagaagctgaagaagatcagcaaccaggccgagttcatcgccagcttctacaagaacgacctgatcaagatcaacggcgagctgtacagggtgatcggcgtgaacaacgacctgctgaacaggatcgaggtgaacatgatcgacatcacctacagggagtacctggagaacatgaacgacaagaggcctcctcacatcatcaagaccatcgccagcaagacccagagcatcaagaagtacagcaccgacatcctgggcaacctgtacgaggtgaagagcaagaagcaccctcagatcatcaagaagggcggcagcagcggcggcagcaccaacctgagcgacatcatcgagaaggagaccggtaagcaactggttatccaggaatccatcctcatgctcccagaggaggtggaagaagtcattgggaacaagccggaaagcgatatactcgtgcacaccgcctacgacgagagcaccgacgagaatgtcatgcttctgactagcgacgcccctgaatacaagccttgggctctggtcatacaggatagcaacggtgagaacaagattaagatgctctctggtggttctcccaagaagaagaggaaagtctaatagcaataaaggatcgtttattttcattggaagcgtgtgttggttttttgatcaggcgcggagggcctatttcccatgattccttcatatttgcatatacgatacaaggctgttagagagataattagaattaatttgactgtaaacacaaagatattagtacaaaatacgtgacgtagaaagtaataatttcttgggtagtttgcagttttaaaattatgttttaaaatggactatcatatgcttaccgtaacttgaaagtatttcgatttcttggctttatatatcttgtggaaaggacgaaacaccgcattatttttctgtaagaccgttatagtactctggaaacagaatctactataacaaggcaaaatgccgtgtttatctcgtcaacttgttggcgagattttttttttttttctagaccgcggccgc

SEQ ID NO: 7 - DNA, 20 bp, Artificial Sequence
  sgRNA targeting the human DMD gene Exon50
acttacaggctccaatagtg

SEQ ID NO: 8 - DNA, 20 bp, Artificial Sequence
  sgRNA-1 targeting the human DMD gene Exon51
gtaacagtctgagtaggagc

SEQ ID NO: 9 - DNA, 20 bp, Artificial Sequence
  sgRNA-2 targeting the human DMD gene Exon51
tgtgtcaccagagtaacagt

SEQ ID NO: 10 - DNA, 20 bp, Artificial Sequence
  sgRNA-3 targeting the human DMD gene Exon51
gtaaccacaggttgtgtcac

SEQ ID NO: 11 - DNA, 20 bp, Artificial Sequence
  sgRNA-4 targeting the human DMD gene Exon51
gctcctactcagactgttac

SEQ ID NO: 12 - DNA, 20 bp, Artificial Sequence
  sgRNA-5 targeting the human DMD gene Exon51
gttactctggtgacacaacc

SEQ ID NO: 13 - DNA, 20 bp, Artificial Sequence
  sgRNA-6 targeting the human DMD gene Exon51
tggcagtttccttagtaacc

SEQ ID NO: 14 - DNA, 20 bp, Artificial Sequence
  sgRNA-7 targeting the human DMD gene Exon51
caggtacctccaacatcaag

SEQ ID NO: 15 - DNA, 20 bp, Artificial Sequence
  sgRNA-8 targeting the human DMD gene Exon51
gaaactgccatctccaaact

SEQ ID NO: 16 - DNA, 20 bp, Artificial Sequence
  sgRNA-9 targeting the human DMD gene Exon51
tgatcaagcagagaaagcca

SEQ ID NO: 17 - DNA, 20 bp, Artificial Sequence
  sgRNA-10 targeting the human DMD gene Exon51
aacttgatcaagcagagaaa

SEQ ID NO: 18 - DNA, 20 bp, Artificial Sequence
  sgRNA-11 targeting the human DMD gene Exon51
aaggtatgagaaaaaatgat

SEQ ID NO: 19 - DNA, 20 bp, Artificial Sequence
  sgRNA-12 targeting the human DMD gene Exon51 acaggttgtgtcaccagagt
acaggttgtgtcaccagagt

SEQ ID NO: 20 - DNA, 20 bp, Artificial Sequence
  sgRNA-13 targeting the human DMD gene Exon51
aacgagatgatcatcaagca

SEQ ID NO: 21 - DNA, 30 bp, Homo sapiens
ctgttactctggtgacacaacctgtggtta

SEQ ID NO: 22 - DNA, 30 bp, Homo sapiens
agactgttactctggtgacacaacctgtgg

SEQ ID NO: 23 - DNA, 30 bp, Homo sapiens
tcttccttgatgttggaggtacctgctctg

SEQ ID NO: 24 - DNA, 30 bp, Homo sapiens
atatcaacgagatgatcatcaagcagaagg